European Patent Specification EP 3 660 852 B1, published May 1, 2024. Title: 一种基于免疫算法的密码子优化方法. The sequence listing filed with the application follows.

SEQUENCE LISTING (6 sequences)

SEQ ID NO: 1 - protein, 430 aa, 人工序列
  JNK3蛋白序列
MSLHFLYYCSEPTLDVKIAFCQGFDKQVDVSYIAKHYNMSKSKVDNQFYSVEVGDSTFTVLKRYQNLKPIGSGAQGIVCAAYDAVLDRNVAIKKLSRPFQNQTHAKRAYRELVLMKCVNHKNIISLLNVFTPQKTLEEFQDVYLVMELMDANLCQVIQMELDHERMSYLLYQMLCGIKHLHSAGIIHRDLKPSNIVVKSDCTLKILDFGLARTAGTSFMMTPYVVTRYYRAPEVILGMGYKENVDIWSVGCIMGEMVRHKILFPGRDYIDQWNKVIEQLGTPCPEFMKKLQPTVRNYVENRPKYAGLTFPKLFPDSLFPADSEHNKLKASQARDLLSKMLVIDPAKRISVDDALQHPYINVWYDPAEVEAPPPQIYDKQLDEREHTIEEWKELIYKEVMNSEEKTKNGVVKGQPSPSAQVQQDYKDDDDK

SEQ ID NO: 2 - protein, 246 aa, 人工序列
  GFP蛋白序列
MSKGEELFTGVVPILVELDGDVNGQKFSVSGEGEGDATYGKLTLKFICTTGKLPVPWPTLVTTFSYGVQCFSRYPDHMKQHDFFKSAMPEGYVQERTIFYKDDGNYKTRAEVKFEGDTLVNRIELKGIDFKEDGNILGHKMEYNYNSHNVYIMADKPKNGIKVNFKIRHNIKDGSVQLADHYQQNTPIGDGPVLLPDNHYLSTQSALSKDPNEKRDHMILLEFVTAAGITHGMDELYKDYKDDDDK

SEQ ID NO: 3 - DNA, 1290 bp, 人工序列
  优化前JNK3蛋白编码序列
atgagcctccatttcttatactactgcagtgaaccaacattggatgtgaaaattgccttttgtcagggattcgataaacaagtggatgtgtcatatattgccaaacattacaacatgagcaaaagcaaagttgacaaccagttctacagtgtggaagtgggagactcaaccttcacagttctcaagcgctaccagaatctaaagcctattggctctggggctcagggcatagtttgtgccgcgtatgatgctgtccttgacagaaatgtggccattaagaagctcagcagaccctttcagaaccaaacacatgccaagagagcgtaccgggagctggtcctcatgaagtgtgtgaaccataaaaacattattagtttattaaatgtcttcacaccccagaaaacgctggaggagttccaagatgtttacttagtaatggaactgatggatgccaacttatgtcaagtgattcagatggaattagaccatgagcgaatgtcttacctgctgtaccaaatgttgtgtggcattaagcacctccattctgctggaattattcacagggatttaaaaccaagtaacattgtagtcaagtctgattgcacattgaaaatcctggactttggactggccaggacagcaggcacaagcttcatgatgactccatatgtggtgacacgttattacagagcccctgaggtcatcctggggatgggctacaaggagaacgtggatatatggtctgtgggatgcattatgggagaaatggttcgccacaaaatcctctttccaggaagggactatattgaccagtggaataaggtaattgaacaactaggaacaccatgtccagaattcatgaagaaattgcaacccacagtaagaaactatgtggagaatcggcccaagtatgcgggactcaccttccccaaactcttcccagattccctcttcccagcggactccgagcacaataaactcaaagccagccaagccagggacttgttgtcaaagatgctagtgattgacccagcaaaaagaatatcagtggacgacgccttacagcatccctacatcaacgtctggtatgacccagccgaagtggaggcgcctccacctcagatatatgacaagcagttggatgaaagagaacacacaattgaagaatggaaagaacttatctacaaggaagtaatgaattcagaagaaaagactaaaaatggtgtagtaaaaggacagccttctccttcagcacaggtgcagcaggactacaaggatgatgatgacaaa

SEQ ID NO: 4 - DNA, 738 bp, 人工序列
  优化前GFP蛋白编码序列
atgagtaaaggagaagaacttttcactggagttgtcccaattcttgttgaattagatggcgatgttaatgggcaaaaattctctgtcagtggagagggtgaaggtgatgcaacatacggaaaacttacccttaaatttatttgcactactgggaagctacctgttccatggccaacacttgtcactactttctcttatggtgttcaatgcttttcaagatacccagatcatatgaaacagcatgactttttcaagagtgccatgcccgaaggttatgtacaggaaagaactatattttacaaagatgacgggaactacaagacacgtgctgaagtcaagtttgaaggtgatacccttgttaatagaatcgagttaaaaggtattgattttaaagaagatggaaacattcttggacacaaaatggaatacaactataactcacataatgtatacatcatggcagacaaaccaaagaatggaatcaaagttaacttcaaaattagacacaacattaaagatggaagcgttcaattagcagaccattatcaacaaaatactccaattggcgatggccctgtccttttaccagacaaccattacctgtccacacaatctgccctttccaaagatcccaacgaaaagagagatcacatgatccttcttgagtttgtaacagctgctgggattacacatggcatggatgaactatacaaagactacaaagatgatgatgacaag

SEQ ID NO: 5 - DNA, 1290 bp, 人工序列
  优化后JNK3蛋白编码序列
atgtctctgcacttcctgtactactgttctgagcccaccctggacgtgaagattgccttctgccagggctttgacaagcaggtggatgtgagctacatcgccaagcactacaacatgtccaagagcaaggtggacaaccagttctacagcgtggaggtgggagacagcaccttcacagtgctgaagagataccagaacctgaagccaattggctctggagcccagggcattgtgtgtgctgcctatgatgctgtgctggacagaaatgtggccatcaagaagctgagcagacccttccagaaccagacacatgccaagagagcctacagagagctggtgctgatgaagtgtgtgaaccacaagaacatcatcagcctgctgaatgtgttcacccctcagaagacactggaggagttccaggatgtgtacctggtgatggagctcatggatgccaacctgtgccaggtgatccagatggagctggaccatgagaggatgagctacctgctgtaccagatgctgtgtggcatcaagcacctgcacagtgctggaatcatccacagagacctgaagccaagcaacattgtggtgaagtctgactgtacactgaagatcctggactttggactggccagaacagccggcacatcttttatgatgacaccatacgtggtgacaagatactacagagcccctgaggtgatcctgggcatgggctacaaggagaacgtggacatctggtctgtgggctgcatcatgggagagatggtgagacacaagatcctgtttcctggaagagactacattgaccagtggaacaaggtgattgagcagctgggcaccccttgtcctgagttcatgaagaagctgcagccaactgtgaggaactatgtggagaacagaccaaagtatgctggcctgaccttccccaagctcttccctgacagcctgtttcctgctgattctgagcacaacaagctgaaggccagccaggccagagacctgctgagcaagatgctggtgattgatcctgccaagagaatctctgtggatgatgccctgcagcacccctacatcaatgtgtggtacgacccagctgaggtggaggccccacctccacagatctatgacaagcagctggatgagagagagcacacaattgaagagtggaaggagctgatctacaaagaagtgatgaactctgaggagaagaccaagaatggagtggtgaagggccagccctctccaagcgcccaggtgcagcaggactacaaggatgatgatgacaaa

SEQ ID NO: 6 - DNA, 738 bp, 人工序列
  优化后GFP蛋白编码序列
atgagcaagggagaggaactgttcacaggagtggtgcccatcctggtggagctggatggagatgtgaatggccagaagttttctgtgtctggggaaggagaaggcgatgccacctatggcaagctgacactgaagttcatctgcaccacagggaagctgcctgtgccctggccaacactggtgaccaccttctcctatggagtccagtgcttcagcagatacccagaccacatgaagcagcatgacttcttcaagagtgccatgcctgagggctatgtgcaggagagaaccatcttctataaggatgatggaaactacaagacaagagctgaggtgaagtttgagggagacaccctggtgaacagaattgagctgaagggcattgacttcaaggaggatggcaacatcctgggccacaagatggagtacaattacaacagccacaatgtgtacatcatggctgataagccaaagaatggaatcaaggtgaacttcaagattagacacaacatcaaagacggatctgtgcagctggctgaccattaccagcagaacacacccattggagatggcccagtgctgctgcccgacaaccactacctgagcacacagtctgccctgagtaaggaccctaatgagaagagggaccacatgattctgctggagtttgtgacagctgctggcatcacccatggcatggatgagctgtacaaggactacaaagatgatgatgacaag